European Patent Application EP 4 389 909 A1, published June 26, 2024. Title: NOVEL SENSOR. Applicant: ESYA LIMITED. The sequence listing filed with the application follows.

SEQUENCE LISTING (6 sequences)

SEQ ID NO: 1 - protein, 8 aa, synthetic construct
EVNLDAEF

SEQ ID NO: 2 - DNA, 41 bp, synthetic construct
  source 1..41: mol_type = other DNA
ataacacataacacataacaaaatatatatcctagaacgac

SEQ ID NO: 3 - DNA, 42 bp, synthetic construct
  source 1..42: mol_type = other DNA
tgtcgttctaggatatatattttgttatgtgttatgtgttat

SEQ ID NO: 4 - DNA, 41 bp, synthetic construct
  source 1..41: mol_type = other DNA
gtcgttctaggatatatattttgttatgtgttatgtgttat

SEQ ID NO: 5 - protein, 10 aa, synthetic construct
RKFEADLNVE

SEQ ID NO: 6 - protein, 10 aa, synthetic construct
KFEADLNVEK